European Patent Application EP 4 183 451 A1, published May 24, 2023. Title: COMPOSITIONS AND METHODS FOR ADJOINING TYPE I AND TYPE II EXTRACELLULAR DOMAINS AS HETEROLOGOUS CHIMERIC PROTEINS. Applicant: Heat Biologics, Inc. The sequence listing filed with the application follows.

SEQUENCE LISTING (78 sequences)

SEQ ID NO: 1 - DNA, 1605 bp, synthetic construct
  misc_feature 1..1605: note = Synthetic sequence
  source 1..1605: mol_type = other DNA
atgcagatcccacaggcgccctggccagtcgtctgggcggtgctacaactgggctggcggccaggatggttcttagactccccagacaggccctggaacccccccaccttctccccagccctgctcgtggtgaccgaaggggacaacgccaccttcacctgcagcttctccaacacatcggagagcttcgtgctaaactggtaccgcatgagccccagcaaccagacggacaagctggccgccttccccgaggaccgcagccagcccggccaggactgccgcttccgtgtcacacaactgcccaacgggcgtgacttccacatgagcgtggtcagggcccggcgcaatgacagcggcacctacctctgtggggccatctccctggcccccaaggcgcagatcaaagagagcctgcgggcagagctcagggtgacagagagaagggcagaagtgcccacagcccaccccagcccctcacccaggccagccggccagttccaatctaagtacggccctccctgccctagctgtcccgcccctgaatttctgggcggaccctccgtgtttctgttccccccaaagcccaaggacaccctgatgatcagccggacccccgaagtgacctgtgtggtggtggatgtgtcccaggaagatcccgaggtgcagttcaattggtacgtggacggggtggaagtgcacaacgccaagaccaagcccagagaggaacagttcaacagcacctaccgggtggtgtctgtgctgaccgtgctgcaccaggattggctgagcggcaaagagtacaagtgcaaggtgtccagcaagggcctgcccagcagcatcgaaaagaccatcagcaacgccaccggccagcccagggaaccccaggtgtacacactgccccctagccaggaagagatgaccaagaaccaggtgtccctgacatgcctcgtgaagggcttctacccctccgatatcgccgtggaatgggagagcaacggccagccagagaacaactacaagaccacccccccagtgctggacagcgacggctcattcttcctgtactcccggctgacagtggacaagagcagctggcaggaaggcaacgtgttcagctgcagcgtgatgcacgaagccctgcacaaccactacacccagaagtccctgagcctgtccctgggcaaaatagagggacgaatggaccaggtatcacatcggtatcctcgaattcaaagtatcaaagtacaatttaccgaatataagaaggagaaaggtttcatcctcacttcccaaaaggaggatgaaatcatgaaggtgcagaacaactcagtcatcatcaactgtgatgggttttatctcatctccctgaagggctacttctcccaggaagtcaacattagccttcattaccagaaggatgaggagcccctcttccaactgaagaaggtcaggtctgtcaactccttgatggtggcctctctgacttacaaagacaaagtctacttgaatgtgaccactgacaatacctccctggatgacttccatgtgaatggcggagaactgattcttatccatcaaaatcctggtgaattctgtgtcctttga

SEQ ID NO: 2 - protein, 534 aa, synthetic construct
  REGION 1..534: note = Synthetic sequence
MQIPQAPWPVVWAVLQLGWRPGWFLDSPDRPWNPPTFSPALLVVTEGDNATFTCSFSNTSESFVLNWYRMSPSNQTDKLAAFPEDRSQPGQDCRFRVTQLPNGRDFHMSVVRARRNDSGTYLCGAISLAPKAQIKESLRAELRVTERRAEVPTAHPSPSPRPAGQFQSKYGPPCPSCPAPEFLGGPSVFLFPPKPKDTLMISRTPEVTCVVVDVSQEDPEVQFNWYVDGVEVHNAKTKPREEQFNSTYRVVSVLTVLHQDWLSGKEYKCKVSSKGLPSSIEKTISNATGQPREPQVYTLPPSQEEMTKNQVSLTCLVKGFYPSDIAVEWESNGQPENNYKTTPPVLDSDGSFFLYSRLTVDKSSWQEGNVFSCSVMHEALHNHYTQKSLSLSLGKIEGRMDQVSHRYPRIQSIKVQFTEYKKEKGFILTSQKEDEIMKVQNNSVIINCDGFYLISLKGYFSQEVNISLHYQKDEEPLFQLKKVRSVNSLMVASLTYKDKVYLNVTTDNTSLDDFHVNGGELILIHQNPGEFCVL

SEQ ID NO: 3 - DNA, 1782 bp, synthetic construct
  misc_feature 1..1782: note = Synthetic sequence
  source 1..1782: mol_type = other DNA
atgcagattcctcaggccccttggcctgtcgtgtgggctgtgctgcagctgggatggcggcctggctggtttctggacagccccgacagaccctggaacccccctacattttcccctgccctgctggtcgtgaccgagggcgacaatgccaccttcacctgtagcttcagcaacaccagcgagagcttcgtgctgaactggtacagaatgagccccagcaaccagaccgacaagctggccgccttccccgaggatagatctcagcccggccaggactgccggttcagagtgacccagctgcccaacggccgggacttccacatgtctgtcgtgcgggccagacggaacgacagcggcacatatctgtgcggcgccatcagcctggcccccaaggcccagatcaaagagagcctgagagccgagctgagagtgaccgagagaagggccgaagtgcctaccgcccaccctagcccatctccaagacctgccggccagttccagtctaagtacggccctccttgccccagctgtcccgcccctgaatttctgggcggacccagcgtgttcctgttccccccaaagcccaaggacaccctgatgatcagccggacccccgaagtgacctgcgtggtggtggatgtgtcccaggaagatcccgaggtgcagttcaattggtacgtggacggcgtggaagtgcacaacgccaagaccaagcccagagaggaacagttcaacagcacctaccgggtggtgtccgtgctgaccgtgctgcaccaggattggctgagcggcaaagagtacaagtgcaaggtgtccagcaagggcctgcccagcagcatcgagaaaaccatcagcaacgccaccggccagcccagggaaccccaggtgtacacactgccccctagccaggaagagatgaccaagaaccaggtgtccctgacctgtctcgtgaagggcttctacccctccgatatcgccgtggaatgggagagcaacggccagcctgagaacaactacaagaccacccccccagtgctggacagcgacggctcatttttcctgtactccagactgaccgtggacaagagcagctggcaggaaggcaacgtgttcagctgctccgtgatgcacgaggccctgcacaaccactacacccagaagtccctgtctctgagcctgggcaagatcgagggccggatggatagagcccagggcgaagcctgcgtgcagttccaggctctgaagggccaggaattcgcccccagccaccagcaggtgtacgcccctctgagagctgacggcgacaagcctagagcccacctgacagtcgtgcggcagacccctacccagcacttcaagaatcagttcccagccctgcactgggagcacgagctgggcctggccttcaccaagaacagaatgaactacaccaacaagtttctgctgatccccgagagcggcgactacttcatctacagccaagtgaccttccggggcatgaccagcgagtgcagcgagatcagacaggccggcagacctaacaagcccgacagcatcaccgtcgtgatcaccaaagtgaccgacagctaccccgagcccacacagctgctgatgggcaccaagagcgtgtgcgaagtgggcagcaactggttccagcccatctacctgggcgccatgttcagtctgcaagagggcgataagctgatggtcaacgtgtccgacatctccctggtggattacaccaaagaggacaagaccttcttcggcgcctttctgctctga

SEQ ID NO: 4 - DNA, 1782 bp, synthetic construct
  misc_feature 1..1782: note = Synthetic sequence
  source 1..1782: mol_type = other DNA
atgcagatcccacaggcgccctggccagtcgtctgggcggtgctacaactgggctggcggccaggatggttcttagactccccagacaggccctggaacccccccaccttctccccagccctgctcgtggtgaccgaaggggacaacgccaccttcacctgcagcttctccaacacatcggagagcttcgtgctaaactggtaccgcatgagccccagcaaccagacggacaagctggccgccttccccgaggaccgcagccagcccggccaggactgccgcttccgtgtcacacaactgcccaacgggcgtgacttccacatgagcgtggtcagggcccggcgcaatgacagcggcacctacctctgtggggccatctccctggcccccaaggcgcagatcaaagagagcctgcgggcagagctcagggtgacagagagaagggcagaagtgcccacagcccaccccagcccctcacccaggccagccggccagttccaatctaagtacggccctccctgccctagctgtcccgcccctgaatttctgggcggaccctccgtgtttctgttccccccaaagcccaaggacaccctgatgatcagccggacccccgaagtgacctgtgtggtggtggatgtgtcccaggaagatcccgaggtgcagttcaattggtacgtggacggggtggaagtgcacaacgccaagaccaagcccagagaggaacagttcaacagcacctaccgggtggtgtctgtgctgaccgtgctgcaccaggattggctgagcggcaaagagtacaagtgcaaggtgtccagcaagggcctgcccagcagcatcgaaaagaccatcagcaacgccaccggccagcccagggaaccccaggtgtacacactgccccctagccaggaagagatgaccaagaaccaggtgtccctgacatgcctcgtgaagggcttctacccctccgatatcgccgtggaatgggagagcaacggccagccagagaacaactacaagaccacccccccagtgctggacagcgacggctcattcttcctgtactcccggctgacagtggacaagagcagctggcaggaaggcaacgtgttcagctgcagcgtgatgcacgaagccctgcacaaccactacacccagaagtccctgagcctgtccctgggcaaaatagagggacgaatggaccgggcccagggagaggcctgtgtgcagttccaggctctaaaaggacaggagtttgcaccttcacatcagcaagtttatgcacctcttagagcagacggagataagccaagggcacacctgacagttgtgagacaaactcccacacagcactttaaaaatcagttcccagctctgcactgggaacatgaactaggcctggccttcaccaagaaccgaatgaactataccaacaaattcctgctgatcccagagtcgggagactacttcatttactcccaggtcacattccgtgggatgacctctgagtgcagtgaaatcagacaagcaggccgaccaaacaagccagactccatcactgtggtcatcaccaaggtaacagacagctaccctgagccaacccagctcctcatggggaccaagtctgtatgcgaagtaggtagcaactggttccagcccatctacctcggagccatgttctccttgcaagaaggggacaagctaatggtgaacgtcagtgacatctctttggtggattacacaaaagaagataaaaccttctttggagccttcttactatag

SEQ ID NO: 5 - protein, 593 aa, synthetic construct
  REGION 1..593: note = Synthetic sequence
MQIPQAPWPVVWAVLQLGWRPGWFLDSPDRPWNPPTFSPALLVVTEGDNATFTCSFSNTSESFVLNWYRMSPSNQTDKLAAFPEDRSQPGQDCRFRVTQLPNGRDFHMSVVRARRNDSGTYLCGAISLAPKAQIKESLRAELRVTERRAEVPTAHPSPSPRPAGQFQSKYGPPCPSCPAPEFLGGPSVFLFPPKPKDTLMISRTPEVTCVVVDVSQEDPEVQFNWYVDGVEVHNAKTKPREEQFNSTYRVVSVLTVLHQDWLSGKEYKCKVSSKGLPSSIEKTISNATGQPREPQVYTLPPSQEEMTKNQVSLTCLVKGFYPSDIAVEWESNGQPENNYKTTPPVLDSDGSFFLYSRLTVDKSSWQEGNVFSCSVMHEALHNHYTQKSLSLSLGKIEGRMDRAQGEACVQFQALKGQEFAPSHQQVYAPLRADGDKPRAHLTVVRQTPTQHFKNQFPALHWEHELGLAFTKNRMNYTNKFLLIPESGDYFIYSQVTFRGMTSECSEIRQAGRPNKPDSITVVITKVTDSYPEPTQLLMGTKSVCEVGSNWFQPIYLGAMFSLQEGDKLMVNVSDISLVDYTKEDKTFFGAFLL

SEQ ID NO: 6 - DNA, 1554 bp, synthetic construct
  misc_feature 1..1554: note = Synthetic sequence
  source 1..1554: mol_type = other DNA
atgaagacattgcctgccatgcttggaactgggaaattattttgggtcttcttcttaatcccatatctggacatctggaacatccatgggaaagaatcatgtgatgtacagctttatataaagagacaatctgaacactccatcttagcaggagatccctttgaactagaatgccctgtgaaatactgtgctaacaggcctcatgtgacttggtgcaagctcaatggaacaacatgtgtaaaacttgaagatagacaaacaagttggaaggaagagaagaacatttcatttttcattctacattttgaaccagtgcttcctaatgacaatgggtcataccgctgttctgcaaattttcagtctaatctcattgaaagccactcaacaactctttatgtgacagatgtaaaaagtgcctcagaacgaccctccaaggacgaaatggcaagctctaagtacggccctccctgccctagctgtcccgcccctgaatttctgggcggaccctccgtgtttctgttccccccaaagcccaaggacaccctgatgatcagccggacccccgaagtgacctgtgtggtggtggatgtgtcccaggaagatcccgaggtgcagttcaattggtacgtggacggggtggaagtgcacaacgccaagaccaagcccagagaggaacagttcaacagcacctaccgggtggtgtctgtgctgaccgtgctgcaccaggattggctgagcggcaaagagtacaagtgcaaggtgtccagcaagggcctgcccagcagcatcgaaaagaccatcagcaacgccaccggccagcccagggaaccccaggtgtacacactgccccctagccaggaagagatgaccaagaaccaggtgtccctgacatgcctcgtgaagggcttctacccctccgatatcgccgtggaatgggagagcaacggccagccagagaacaactacaagaccacccccccagtgctggacagcgacggctcattcttcctgtactcccggctgacagtggacaagagcagctggcaggaaggcaacgtgttcagctgcagcgtgatgcacgaagccctgcacaaccactacacccagaagtccctgagcctgtccctgggcaaaatagagggacgaatggaccaggtatcacatcggtatcctcgaattcaaagtatcaaagtacaatttaccgaatataagaaggagaaaggtttcatcctcacttcccaaaaggaggatgaaatcatgaaggtgcagaacaactcagtcatcatcaactgtgatgggttttatctcatctccctgaagggctacttctcccaggaagtcaacattagccttcattaccagaaggatgaggagcccctcttccaactgaagaaggtcaggtctgtcaactccttgatggtggcctctctgacttacaaagacaaagtctacttgaatgtgaccactgacaatacctccctggatgacttccatgtgaatggcggagaactgattcttatccatcaaaatcctggtgaattctgtgtcctttga

SEQ ID NO: 7 - protein, 517 aa, synthetic construct
  REGION 1..517: note = Synthetic sequence
MKTLPAMLGTGKLFWVFFLIPYLDIWNIHGKESCDVQLYIKRQSEHSILAGDPFELECPVKYCANRPHVTWCKLNGTTCVKLEDRQTSWKEEKNISFFILHFEPVLPNDNGSYRCSANFQSNLIESHSTTLYVTDVKSASERPSKDEMASSKYGPPCPSCPAPEFLGGPSVFLFPPKPKDTLMISRTPEVTCVVVDVSQEDPEVQFNWYVDGVEVHNAKTKPREEQFNSTYRVVSVLTVLHQDWLSGKEYKCKVSSKGLPSSIEKTISNATGQPREPQVYTLPPSQEEMTKNQVSLTCLVKGFYPSDIAVEWESNGQPENNYKTTPPVLDSDGSFFLYSRLTVDKSSWQEGNVFSCSVMHEALHNHYTQKSLSLSLGKIEGRMDQVSHRYPRIQSIKVQFTEYKKEKGFILTSQKEDEIMKVQNNSVIINCDGFYLISLKGYFSQEVNISLHYQKDEEPLFQLKKVRSVNSLMVASLTYKDKVYLNVTTDNTSLDDFHVNGGELILIHQNPGEFCVL

SEQ ID NO: 8 - DNA, 1527 bp, synthetic construct
  misc_feature 1..1527: note = Synthetic sequence
  source 1..1527: mol_type = other DNA
atgcgctggtgtctcctcctgatctgggcccaggggctgaggcaggctcccctcgcctcaggaatgatgacaggcacaatagaaacaacggggaacatttctgcagagaaaggtggctctatcatcttacaatgtcacctctcctccaccacggcacaagtgacccaggtcaactgggagcagcaggaccagcttctggccatttgtaatgctgacttggggtggcacatctccccatccttcaaggatcgagtggccccaggtcccggcctgggcctcaccctccagtcgctgaccgtgaacgatacaggggagtacttctgcatctatcacacctaccctgatgggacgtacactgggagaatcttcctggaggtcctagaaagctcagtggctgagcacggtgccaggttccagattccatctaagtacggccctccctgccctagctgtcccgcccctgaatttctgggcggaccctccgtgtttctgttccccccaaagcccaaggacaccctgatgatcagccggacccccgaagtgacctgtgtggtggtggatgtgtcccaggaagatcccgaggtgcagttcaattggtacgtggacggggtggaagtgcacaacgccaagaccaagcccagagaggaacagttcaacagcacctaccgggtggtgtctgtgctgaccgtgctgcaccaggattggctgagcggcaaagagtacaagtgcaaggtgtccagcaagggcctgcccagcagcatcgaaaagaccatcagcaacgccaccggccagcccagggaaccccaggtgtacacactgccccctagccaggaagagatgaccaagaaccaggtgtccctgacatgcctcgtgaagggcttctacccctccgatatcgccgtggaatgggagagcaacggccagccagagaacaactacaagaccacccccccagtgctggacagcgacggctcattcttcctgtactcccggctgacagtggacaagagcagctggcaggaaggcaacgtgttcagctgcagcgtgatgcacgaagccctgcacaaccactacacccagaagtccctgagcctgtccctgggcaaaatagagggacgaatggaccaggtatcacatcggtatcctcgaattcaaagtatcaaagtacaatttaccgaatataagaaggagaaaggtttcatcctcacttcccaaaaggaggatgaaatcatgaaggtgcagaacaactcagtcatcatcaactgtgatgggttttatctcatctccctgaagggctacttctcccaggaagtcaacattagccttcattaccagaaggatgaggagcccctcttccaactgaagaaggtcaggtctgtcaactccttgatggtggcctctctgacttacaaagacaaagtctacttgaatgtgaccactgacaatacctccctggatgacttccatgtgaatggcggagaactgattcttatccatcaaaatcctggtgaattctgtgtcctttga

SEQ ID NO: 9 - protein, 508 aa, synthetic construct
  REGION 1..508: note = Synthetic sequence
MRWCLLLIWAQGLRQAPLASGMMTGTIETTGNISAEKGGSIILQCHLSSTTAQVTQVNWEQQDQLLAICNADLGWHISPSFKDRVAPGPGLGLTLQSLTVNDTGEYFCIYHTYPDGTYTGRIFLEVLESSVAEHGARFQIPSKYGPPCPSCPAPEFLGGPSVFLFPPKPKDTLMISRTPEVTCVVVDVSQEDPEVQFNWYVDGVEVHNAKTKPREEQFNSTYRVVSVLTVLHQDWLSGKEYKCKVSSKGLPSSIEKTISNATGQPREPQVYTLPPSQEEMTKNQVSLTCLVKGFYPSDIAVEWESNGQPENNYKTTPPVLDSDGSFFLYSRLTVDKSSWQEGNVFSCSVMHEALHNHYTQKSLSLSLGKIEGRMDQVSHRYPRIQSIKVQFTEYKKEKGFILTSQKEDEIMKVQNNSVIINCDGFYLISLKGYFSQEVNISLHYQKDEEPLFQLKKVRSVNSLMVASLTYKDKVYLNVTTDNTSLDDFHVNGGELILIHQNPGEFCVL

SEQ ID NO: 10 - DNA, 1710 bp, synthetic construct
  misc_feature 1..1710: note = Synthetic sequence
  source 1..1710: mol_type = other DNA
atgttttcacatcttccctttgactgtgtcctgctgctgctgctgctactacttacaaggtcctcagaagtggaatacagagcggaggtcggtcagaatgcctatctgccctgcttctacaccccagccgccccagggaacctcgtgcccgtctgctggggcaaaggagcctgtcctgtgtttgaatgtggcaacgtggtgctcaggactgatgaaagggatgtgaattattggacatccagatactggctaaatggggatttccgcaaaggagatgtgtccctgaccatagagaatgtgactctagcagacagtgggatctactgctgccggatccaaatcccaggcataatgaatgatgaaaaatttaacctgaagttggtcatcaaaccagccaaggtcacccctgcaccgactcggcagagagacttcactgcagcctttccaaggatgcttaccaccaggggacatggcccagcagagacacagacactggggagcctccctgatataaatctaacacaaatatccacattggccaatgagttacgggactctagattggccaatgacttacgggactctggagcaaccatcagaataggctctaagtacggccctccctgccctagctgtcccgcccctgaatttctgggcggaccctccgtgtttctgttccccccaaagcccaaggacaccctgatgatcagccggacccccgaagtgacctgtgtggtggtggatgtgtcccaggaagatcccgaggtgcagttcaattggtacgtggacggggtggaagtgcacaacgccaagaccaagcccagagaggaacagttcaacagcacctaccgggtggtgtctgtgctgaccgtgctgcaccaggattggctgagcggcaaagagtacaagtgcaaggtgtccagcaagggcctgcccagcagcatcgaaaagaccatcagcaacgccaccggccagcccagggaaccccaggtgtacacactgccccctagccaggaagagatgaccaagaaccaggtgtccctgacatgcctcgtgaagggcttctacccctccgatatcgccgtggaatgggagagcaacggccagccagagaacaactacaagaccacccccccagtgctggacagcgacggctcattcttcctgtactcccggctgacagtggacaagagcagctggcaggaaggcaacgtgttcagctgcagcgtgatgcacgaagccctgcacaaccactacacccagaagtccctgagcctgtccctgggcaaaatagagggacgaatggaccaggtatcacatcggtatcctcgaattcaaagtatcaaagtacaatttaccgaatataagaaggagaaaggtttcatcctcacttcccaaaaggaggatgaaatcatgaaggtgcagaacaactcagtcatcatcaactgtgatgggttttatctcatctccctgaagggctacttctcccaggaagtcaacattagccttcattaccagaaggatgaggagcccctcttccaactgaagaaggtcaggtctgtcaactccttgatggtggcctctctgacttacaaagacaaagtctacttgaatgtgaccactgacaatacctccctggatgacttccatgtgaatggcggagaactgattcttatccatcaaaatcctggtgaattctgtgtcctttga

SEQ ID NO: 11 - protein, 569 aa, synthetic construct
  REGION 1..569: note = Synthetic sequence
MFSHLPFDCVLLLLLLLLTRSSEVEYRAEVGQNAYLPCFYTPAAPGNLVPVCWGKGACPVFECGNVVLRTDERDVNYWTSRYWLNGDFRKGDVSLTIENVTLADSGIYCCRIQIPGIMNDEKFNLKLVIKPAKVTPAPTRQRDFTAAFPRMLTTRGHGPAETQTLGSLPDINLTQISTLANELRDSRLANDLRDSGATIRIGSKYGPPCPSCPAPEFLGGPSVFLFPPKPKDTLMISRTPEVTCVVVDVSQEDPEVQFNWYVDGVEVHNAKTKPREEQFNSTYRVVSVLTVLHQDWLSGKEYKCKVSSKGLPSSIEKTISNATGQPREPQVYTLPPSQEEMTKNQVSLTCLVKGFYPSDIAVEWESNGQPENNYKTTPPVLDSDGSFFLYSRLTVDKSSWQEGNVFSCSVMHEALHNHYTQKSLSLSLGKIEGRMDQVSHRYPRIQSIKVQFTEYKKEKGFILTSQKEDEIMKVQNNSVIINCDGFYLISLKGYFSQEVNISLHYQKDEEPLFQLKKVRSVNSLMVASLTYKDKVYLNVTTDNTSLDDFHVNGGELILIHQNPGEFCVL

SEQ ID NO: 12 - DNA, 2223 bp, synthetic construct
  misc_feature 1..2223: note = Synthetic sequence
  source 1..2223: mol_type = other DNA
atggagcccgccggcccggcccccggccgcctcgggccgctgctctgcctgctgctcgccgcgtcctgcgcctggtcaggagtggcgggtgaggaggagctgcaggtgattcagcctgacaagtccgtgttggttgcagctggagagacagccactctgcgctgcactgcgacctctctgatccctgtggggcccatccagtggttcagaggagctggaccaggccgggaattaatctacaatcaaaaagaaggccacttcccccgggtaacaactgtttcagacctcacaaagagaaacaacatggacttttccatccgcatcggtaacatcaccccagcagatgccggcacctactactgtgtgaagttccggaaagggagccccgatgacgtggagtttaagtctggagcaggcactgagctgtctgtgcgcgccaaaccctctgcccccgtggtatcgggccctgcggcgagggccacacctcagcacacagtgagcttcacctgcgagtcccacggcttctcacccagagacatcaccctgaaatggttcaaaaatgggaatgagctctcagacttccagaccaacgtggaccccgtaggagagagcgtgtcctacagcatccacagcacagccaaggtggtgctgacccgcgaggacgttcactctcaagtcatctgcgaggtggcccacgtcaccttgcagggggaccctcttcgtgggactgccaacttgtctgagaccatccgagttccacccaccttggaggttactcaacagcccgtgagggcagagaaccaggtgaatgtcacctgccaggtgaggaagttctacccccagagactacagctgacctggttggagaatggaaacgtgtcccggacagaaacggcctcaaccgttacagagaacaaggatggtacctacaactggatgagctggctcctggtgaatgtatctgcccacagggatgatgtgaagctcacctgccaggtggagcatgacgggcagccagcggtcagcaaaagccatgacctgaaggtctcagcccacccgaaggagcagggctcaaataccgccgctgagaacactggatctaatgaacggaacatctattctaagtacggccctccctgccctagctgtcccgcccctgaatttctgggcggaccctccgtgtttctgttccccccaaagcccaaggacaccctgatgatcagccggacccccgaagtgacctgtgtggtggtggatgtgtcccaggaagatcccgaggtgcagttcaattggtacgtggacggggtggaagtgcacaacgccaagaccaagcccagagaggaacagttcaacagcacctaccgggtggtgtctgtgctgaccgtgctgcaccaggattggctgagcggcaaagagtacaagtgcaaggtgtccagcaagggcctgcccagcagcatcgaaaagaccatcagcaacgccaccggccagcccagggaaccccaggtgtacacactgccccctagccaggaagagatgaccaagaaccaggtgtccctgacatgcctcgtgaagggcttctacccctccgatatcgccgtggaatgggagagcaacggccagccagagaacaactacaagaccacccccccagtgctggacagcgacggctcattcttcctgtactcccggctgacagtggacaagagcagctggcaggaaggcaacgtgttcagctgcagcgtgatgcacgaagccctgcacaaccactacacccagaagtccctgagcctgtccctgggcaaaatagagggacgaatggaccaggtatcacatcggtatcctcgaattcaaagtatcaaagtacaatttaccgaatataagaaggagaaaggtttcatcctcacttcccaaaaggaggatgaaatcatgaaggtgcagaacaactcagtcatcatcaactgtgatgggttttatctcatctccctgaagggctacttctcccaggaagtcaacattagccttcattaccagaaggatgaggagcccctcttccaactgaagaaggtcaggtctgtcaactccttgatggtggcctctctgacttacaaagacaaagtctacttgaatgtgaccactgacaatacctccctggatgacttccatgtgaatggcggagaactgattcttatccatcaaaatcctggtgaattctgtgtcctttga

SEQ ID NO: 13 - protein, 740 aa, synthetic construct
  REGION 1..740: note = Synthetic sequence
MEPAGPAPGRLGPLLCLLLAASCAWSGVAGEEELQVIQPDKSVLVAAGETATLRCTATSLIPVGPIQWFRGAGPGRELIYNQKEGHFPRVTTVSDLTKRNNMDFSIRIGNITPADAGTYYCVKFRKGSPDDVEFKSGAGTELSVRAKPSAPVVSGPAARATPQHTVSFTCESHGFSPRDITLKWFKNGNELSDFQTNVDPVGESVSYSIHSTAKVVLTREDVHSQVICEVAHVTLQGDPLRGTANLSETIRVPPTLEVTQQPVRAENQVNVTCQVRKFYPQRLQLTWLENGNVSRTETASTVTENKDGTYNWMSWLLVNVSAHRDDVKLTCQVEHDGQPAVSKSHDLKVSAHPKEQGSNTAAENTGSNERNIYSKYGPPCPSCPAPEFLGGPSVFLFPPKPKDTLMISRTPEVTCVVVDVSQEDPEVQFNWYVDGVEVHNAKTKPREEQFNSTYRVVSVLTVLHQDWLSGKEYKCKVSSKGLPSSIEKTISNATGQPREPQVYTLPPSQEEMTKNQVSLTCLVKGFYPSDIAVEWESNGQPENNYKTTPPVLDSDGSFFLYSRLTVDKSSWQEGNVFSCSVMHEALHNHYTQKSLSLSLGKIEGRMDQVSHRYPRIQSIKVQFTEYKKEKGFILTSQKEDEIMKVQNNSVIINCDGFYLISLKGYFSQEVNISLHYQKDEEPLFQLKKVRSVNSLMVASLTYKDKVYLNVTTDNTSLDDFHVNGGELILIHQNPGEFCVL

SEQ ID NO: 14 - DNA, 1554 bp, synthetic construct
  misc_feature 1..1554: note = Synthetic sequence
  source 1..1554: mol_type = other DNA
atggggtccccgggcatggtgctgggcctcctggtgcagatctgggccctgcaagaagcctcaagcctgagcgtgcagcaggggcccaacttgctgcaggtgaggcagggcagtcaggcgaccctggtctgccaggtggaccaggccacagcctgggaacggctccgtgttaagtggacaaaggatggggccatcctgtgtcaaccgtacatcaccaacggcagcctcagcctgggggtctgcgggccccagggacggctctcctggcaggcacccagccatctcaccctgcagctggaccctgtgagcctcaaccacagcggggcgtacgtgtgctgggcggccgtagagattcctgagttggaggaggctgagggcaacataacaaggctctttgtggacccagatgaccccacacagaacagaaaccggatcgcaagcttcccaggatctaagtacggccctccctgccctagctgtcccgcccctgaatttctgggcggaccctccgtgtttctgttccccccaaagcccaaggacaccctgatgatcagccggacccccgaagtgacctgtgtggtggtggatgtgtcccaggaagatcccgaggtgcagttcaattggtacgtggacggggtggaagtgcacaacgccaagaccaagcccagagaggaacagttcaacagcacctaccgggtggtgtctgtgctgaccgtgctgcaccaggattggctgagcggcaaagagtacaagtgcaaggtgtccagcaagggcctgcccagcagcatcgaaaagaccatcagcaacgccaccggccagcccagggaaccccaggtgtacacactgccccctagccaggaagagatgaccaagaaccaggtgtccctgacatgcctcgtgaagggcttctacccctccgatatcgccgtggaatgggagagcaacggccagccagagaacaactacaagaccacccccccagtgctggacagcgacggctcattcttcctgtactcccggctgacagtggacaagagcagctggcaggaaggcaacgtgttcagctgcagcgtgatgcacgaagccctgcacaaccactacacccagaagtccctgagcctgtccctgggcaaaatagagggacgaatggaccaggtatcacatcggtatcctcgaattcaaagtatcaaagtacaatttaccgaatataagaaggagaaaggtttcatcctcacttcccaaaaggaggatgaaatcatgaaggtgcagaacaactcagtcatcatcaactgtgatgggttttatctcatctccctgaagggctacttctcccaggaagtcaacattagccttcattaccagaaggatgaggagcccctcttccaactgaagaaggtcaggtctgtcaactccttgatggtggcctctctgacttacaaagacaaagtctacttgaatgtgaccactgacaatacctccctggatgacttccatgtgaatggcggagaactgattcttatccatcaaaatcctggtgaattctgtgtcctttga

SEQ ID NO: 15 - protein, 517 aa, synthetic construct
  REGION 1..517: note = Synthetic sequence
MGSPGMVLGLLVQIWALQEASSLSVQQGPNLLQVRQGSQATLVCQVDQATAWERLRVKWTKDGAILCQPYITNGSLSLGVCGPQGRLSWQAPSHLTLQLDPVSLNHSGAYVCWAAVEIPELEEAEGNITRLFVDPDDPTQNRNRIASFPGSKYGPPCPSCPAPEFLGGPSVFLFPPKPKDTLMISRTPEVTCVVVDVSQEDPEVQFNWYVDGVEVHNAKTKPREEQFNSTYRVVSVLTVLHQDWLSGKEYKCKVSSKGLPSSIEKTISNATGQPREPQVYTLPPSQEEMTKNQVSLTCLVKGFYPSDIAVEWESNGQPENNYKTTPPVLDSDGSFFLYSRLTVDKSSWQEGNVFSCSVMHEALHNHYTQKSLSLSLGKIEGRMDQVSHRYPRIQSIKVQFTEYKKEKGFILTSQKEDEIMKVQNNSVIINCDGFYLISLKGYFSQEVNISLHYQKDEEPLFQLKKVRSVNSLMVASLTYKDKVYLNVTTDNTSLDDFHVNGGELILIHQNPGEFCVL

SEQ ID NO: 16 - DNA, 3493 bp, Homo sapiens
  source 1..3493: mol_type = genomic DNA
tcaatcgccttttatctctggccctgggacctttgcctattttctgattgataggctttgttttgtctttacctccttctttctggggaaaacttcagttttatcgcacgttccccttttccatatcttcatcttccctctacccagattgtgaagatggaaagggtccaacccctggaagagaatgtgggaaatgcagccaggccaagattcgagaggaacaagctattgctggtggcctctgtaattcagggactggggctgctcctgtgcttcacctacatctgcctgcacttctctgctcttcaggtatcacatcggtatcctcgaattcaaagtatcaaagtacaatttaccgaatataagaaggagaaaggtttcatcctcacttcccaaaaggaggatgaaatcatgaaggtgcagaacaactcagtcatcatcaactgtgatgggttttatctcatctccctgaagggctacttctcccaggaagtcaacattagccttcattaccagaaggatgaggagcccctcttccaactgaagaaggtcaggtctgtcaactccttgatggtggcctctctgacttacaaagacaaagtctacttgaatgtgaccactgacaatacctccctggatgacttccatgtgaatggcggagaactgattcttatccatcaaaatcctggtgaattctgtgtcctttgaggggctgatggcaatatctaaaaccaggcaccagcatgaacaccaagctgggggtggacagggcatggattcttcattgcaagtgaaggagcctcccagctcagccacgtgggatgtgacaagaagcagatcctggccctcccgcccccacccctcagggatatttaaaacttattttatataccagttaatcttatttatccttatattttctaaattgcctagccgtcacaccccaagattgccttgagcctactaggcacctttgtgagaaagaaaaaatagatgcctcttcttcaagatgcattgtttctattggtcaggcaattgtcataataaacttatgtcattgaaaacggtacctgactaccatttgctggaaatttgacatgtgtgtggcattatcaaaatgaagaggagcaaggagtgaaggagtggggttatgaatctgccaaaggtggtatgaaccaacccctggaagccaaagcggcctctccaaggttaaattgattgcagtttgcatattgcctaaatttaaactttctcatttggtgggggttcaaaagaagaatcagcttgtgaaaaatcaggacttgaagagagccgtctaagaaataccacgtgctttttttctttaccattttgctttcccagcctccaaacatagttaatagaaatttcccttcaaagaactgtctggggatgtgatgctttgaaaaatctaatcagtgacttaagagagattttcttgtatacagggagagtgagataacttattgtgaagggttagctttactgtacaggatagcagggaactggacatctcagggtaaaagtcagtacggattttaatagcctggggaggaaaacacattctttgccacagacaggcaaagcaacacatgctcatcctcctgcctatgctgagatacgcactcagctccatgtcttgtacacacagaaacattgctggtttcaagaaatgaggtgatcctattatcaaattcaatctgatgtcaaatagcactaagaagttattgtgccttatgaaaaataatgatctctgtctagaaataccatagaccatatatagtctcacattgataattgaaactagaagggtctataatcagcctatgccagggcttcaatggaatagtatccccttatgtttagttgaaatgtccccttaacttgatataatgtgttatgcttatggcgctgtggacaatctgatttttcatgtcaactttccagatgatttgtaacttctctgtgccaaaccttttataaacataaatttttgagatatgtattttaaaattgtagcacatgtttccctgacattttcaatagaggatacaacatcacagaatctttctggatgattctgtgttatcaaggaattgtactgtgctacaattatctctagaatctccagaaaggtggagggctgttcgcccttacactaaatggtctcagttggatttttttttcctgttttctatttcctcttaagtacaccttcaactatattcccatccctctattttaatctgttatgaaggaaggtaaataaaaatgctaaatagaagaaattgtaggtaaggtaagaggaatcaagttctgagtggctgccaaggcactcacagaatcataatcatggctaaatatttatggagggcctactgtggaccaggcactgggctaaatacttacatttacaagaatcattctgagacagatattcaatgatatctggcttcactactcagaagattgtgtgtgtgtttgtgtgtgtgtgtgtgtgtgtatttcactttttgttattgaccatgttctgcaaaattgcagttactcagtgagtgatatccgaaaaagtaaacgtttatgactataggtaatatttaagaaaatgcatggttcatttttaagtttggaatttttatctatatttctcacagatgtgcagtgcacatgcaggcctaagtatatgttgtgtgtgttgtttgtctttgatgtcatggtcccctctcttaggtgctcactcgctttgggtgcacctggcctgctcttcccatgttggcctctgcaaccacacagggatatttctgctatgcaccagcctcactccaccttccttccatcaaaaatatgtgtgtgtgtctcagtccctgtaagtcatgtccttcacagggagaattaacccttcgatatacatggcagagttttgtgggaaaagaattgaatgaaaagtcaggagatcagaattttaaatttgacttagccactaactagccatgtaaccttgggaaagtcatttcccatttctgggtcttgcttttctttctgttaaatgagaggaatgttaaatatctaacagtttagaatcttatgcttacagtgttatctgtgaatgcacatattaaatgtctatgttcttgttgctatgagtcaaggagtgtaaccttctcctttactatgttgaatgtatttttttctggacaagcttacatcttcctcagccatctttgtgagtccttcaagagcagttatcaattgttagttagatattttctatttagagaatgcttaagggattccaatcccgatccaaatcataatttgttcttaagtatactgggcaggtcccctattttaagtcataattttgtatttagtgctttcctggctctcagagagtattaatattgatattaataatatagttaatagtaatattgctatttacatggaaacaaataaaagatctcagaattcacta

SEQ ID NO: 17 - protein, 183 aa, Homo sapiens
MERVQPLEENVGNAARPRFERNKLLLVASVIQGLGLLLCFTYICLHFSALQVSHRYPRIQSIKVQFTEYKKEKGFILTSQKEDEIMKVQNNSVIINCDGFYLISLKGYFSQEVNISLHYQKDEEPLFQLKKVRSVNSLMVASLTYKDKVYLNVTTDNTSLDDFHVNGGELILIHQNPGEFCVL

SEQ ID NO: 18 - DNA, 684 bp, synthetic construct
  misc_feature 1..684: note = Synthetic sequence
  source 1..684: mol_type = other DNA
tctaagtacggccctccctgccctagctgtcccgcccctgaatttctgggcggaccctccgtgtttctgttccccccaaagcccaaggacaccctgatgatcagccggacccccgaagtgacctgtgtggtggtggatgtgtcccaggaagatcccgaggtgcagttcaattggtacgtggacggggtggaagtgcacaacgccaagaccaagcccagagaggaacagttcaacagcacctaccgggtggtgtctgtgctgaccgtgctgcaccaggattggctgagcggcaaagagtacaagtgcaaggtgtccagcaagggcctgcccagcagcatcgaaaagaccatcagcaacgccaccggccagcccagggaaccccaggtgtacacactgccccctagccaggaagagatgaccaagaaccaggtgtccctgacatgcctcgtgaagggcttctacccctccgatatcgccgtggaatgggagagcaacggccagccagagaacaactacaagaccacccccccagtgctggacagcgacggctcattcttcctgtactcccggctgacagtggacaagagcagctggcaggaaggcaacgtgttcagctgcagcgtgatgcacgaagccctgcacaaccactacacccagaagtccctgagcctgtccctgggcaaa

SEQ ID NO: 19 - DNA, 867 bp, Homo sapiens
  source 1..867: mol_type = genomic DNA
atgcagatcccacaggcgccctggccagtcgtctgggcggtgctacaactgggctggcggccaggatggttcttagactccccagacaggccctggaacccccccaccttctccccagccctgctcgtggtgaccgaaggggacaacgccaccttcacctgcagcttctccaacacatcggagagcttcgtgctaaactggtaccgcatgagccccagcaaccagacggacaagctggccgccttccccgaggaccgcagccagcccggccaggactgccgcttccgtgtcacacaactgcccaacgggcgtgacttccacatgagcgtggtcagggcccggcgcaatgacagcggcacctacctctgtggggccatctccctggcccccaaggcgcagatcaaagagagcctgcgggcagagctcagggtgacagagagaagggcagaagtgcccacagcccaccccagcccctcacccaggccagccggccagttccaaaccctggtggttggtgtcgtgggcggcctgctgggcagcctggtgctgctagtctgggtcctggccgtcatctgctcccgggccgcacgagggacaataggagccaggcgcaccggccagcccctgaaggaggacccctcagccgtgcctgtgttctctgtggactatggggagctggatttccagtggcgagagaagaccccggagccccccgtgccctgtgtccctgagcagacggagtatgccaccattgtctttcctagcggaatgggcacctcatcccccgcccgcaggggctcagctgacggccctcggagtgcccagccactgaggcctgaggatggacactgctcttggcccctctga

SEQ ID NO: 20 - DNA, 1623 bp, synthetic construct
  misc_feature 1..1623: note = Synthetic sequence
  source 1..1623: mol_type = other DNA
gtcgacgccaccatgcagatcccacaggcgccctggccagtcgtctgggcggtgctacaactgggctggcggccaggatggttcttagactccccagacaggccctggaacccccccaccttctccccagccctgctcgtggtgaccgaaggggacaacgccaccttcacctgcagcttctccaacacatcggagagcttcgtgctaaactggtaccgcatgagccccagcaaccagacggacaagctggccgccttccccgaggaccgcagccagcccggccaggactgccgcttccgtgtcacacaactgcccaacgggcgtgacttccacatgagcgtggtcagggcccggcgcaatgacagcggcacctacctctgtggggccatctccctggcccccaaggcgcagatcaaagagagcctgcgggcagagctcagggtgacagagagaagggcagaagtgcccacagcccaccccagcccctcacccaggccagccggccagttccaatctaagtacggccctccctgccctagctgtcccgcccctgaatttctgggcggaccctccgtgtttctgttccccccaaagcccaaggacaccctgatgatcagccggacccccgaagtgacctgtgtggtggtggatgtgtcccaggaagatcccgaggtgcagttcaattggtacgtggacggggtggaagtgcacaacgccaagaccaagcccagagaggaacagttcaacagcacctaccgggtggtgtctgtgctgaccgtgctgcaccaggattggctgagcggcaaagagtacaagtgcaaggtgtccagcaagggcctgcccagcagcatcgaaaagaccatcagcaacgccaccggccagcccagggaaccccaggtgtacacactgccccctagccaggaagagatgaccaagaaccaggtgtccctgacatgcctcgtgaagggcttctacccctccgatatcgccgtggaatgggagagcaacggccagccagagaacaactacaagaccacccccccagtgctggacagcgacggctcattcttcctgtactcccggctgacagtggacaagagcagctggcaggaaggcaacgtgttcagctgcagcgtgatgcacgaagccctgcacaaccactacacccagaagtccctgagcctgtccctgggcaaaatagagggacgaatggaccaggtatcacatcggtatcctcgaattcaaagtatcaaagtacaatttaccgaatataagaaggagaaaggtttcatcctcacttcccaaaaggaggatgaaatcatgaaggtgcagaacaactcagtcatcatcaactgtgatgggttttatctcatctccctgaagggctacttctcccaggaagtcaacattagccttcattaccagaaggatgaggagcccctcttccaactgaagaaggtcaggtctgtcaactccttgatggtggcctctctgacttacaaagacaaagtctacttgaatgtgaccactgacaatacctccctggatgacttccatgtgaatggcggagaactgattcttatccatcaaaatcctggtgaattctgtgtcctttgagtcgac

SEQ ID NO: 21 - DNA, 1637 bp, Homo sapiens
  source 1..1637: mol_type = genomic DNA
caccggcgagatctgccaccatgcagatccctcaggccccctggcctgtcgtgtgggctgtgctgcagctgggatggcggcctggctggttcctggactctcctgacagaccctggaacccccccacctttagccctgctctgctggtcgtgaccgagggcgacaacgccaccttcacctgttccttcagcaacacctccgagtccttcgtgctgaactggtacagaatgtcccccagcaaccagaccgacaagctggccgccttccccgaggatagatcccagcctggacaggactgccggttcagagtgacccagctgcccaacggccgggacttccacatgtctgtcgtgcgggccagacggaacgactccggcacatatctgtgcggcgccatctccctggcccccaaggctcagatcaaagagtctctgcgggccgagctgagagtgaccgagagaagggctgaggtgccaaccgcccaccctagcccatctccaagacctgccggccagttccagtctaagtacggccctccttgccctagctgccctgcccctgaatttctgggcggaccctccgtgttcctgttccccccaaagcccaaggacaccctgatgatctcccggacccccgaagtgacctgcgtggtggtggatgtgtcccaggaagatcccgaggtgcagttcaattggtacgtggacggcgtggaagtgcacaacgccaagaccaagcccagagaggaacagttcaactccacctaccgggtggtgtccgtgctgaccgtgctgcaccaggattggctgtccggcaaagagtacaagtgcaaggtgtcctccaagggcctgccctccagcatcgaaaagaccatctctaacgccaccggccagccccgggaaccccaggtgtacacactgcctccaagccaggaagagatgaccaagaaccaggtgtccctgacctgtctcgtgaagggcttctacccctccgatatcgccgtggaatgggagtccaacggccagcctgagaacaactacaagaccaccccccctgtgctggactccgacggctccttcttcctgtactcccgcctgaccgtggacaagtcctcctggcaggaaggcaacgtgttctcctgctccgtgatgcacgaggccctgcacaaccactacacccagaagtccctgtccctgtctctgggcaagatcgagggccggatggatcaggtgtcacacagatacccccggatccagtccatcaaagtgcagtttaccgagtacaagaaagagaagggattcatcctgacctcccagaaagaggacgagatcatgaaggtgcagaacaactccgtgatcatcaactgcgacgggttctacctgatctccctgaagggctacttcagtcaggaagtgaacatcagcctgcactaccagaaggacgaggaacccctgttccagctgaagaaagtgcggagcgtgaactccctgatggtggcctctctgacctacaaggacaaggtgtacctgaacgtgaccaccgacaatacctccctggacgacttccacgtgaacggcggcgagctgatcctgatccaccagaaccctggcgagttctgcgtgctgtgactcgaggctagc

SEQ ID NO: 22 - protein, 534 aa, synthetic construct; identical to SEQ ID NO: 2
  REGION 1..534: note = Synthetic sequence

SEQ ID NO: 23 - protein, 5 aa, synthetic construct
  REGION 1..5: note = Synthetic sequence
GGGGS

SEQ ID NO: 24 - protein, 5 aa, synthetic construct
  REGION 1..5: note = Synthetic sequence
EAAAK

SEQ ID NO: 25 - protein, 7 aa, synthetic construct
  REGION 1..7: note = Synthetic sequence
AEAAAKA

SEQ ID NO: 26 - protein, 12 aa, synthetic construct
  REGION 1..12: note = Synthetic sequence
AEAAAKEAAAKA

SEQ ID NO: 27 - protein, 46 aa, synthetic construct
  REGION 1..46: note = Synthetic sequence
AEAAAKEAAAKEAAAKEAAAKALEAEAAAKEAAAKEAAAKEAAAKA

SEQ ID NO: 28 - protein, 5 aa, synthetic construct
  REGION 1..5: note = Synthetic sequence
PAPAP

SEQ ID NO: 29 - protein, 18 aa, synthetic construct
  REGION 1..18: note = Synthetic sequence
KESGSVSSEQLAQFRSLD

SEQ ID NO: 30 - protein, 14 aa, synthetic construct
  REGION 1..14: note = Synthetic sequence
EGKSSGSGSESKST

SEQ ID NO: 31 - protein, 12 aa, synthetic construct
  REGION 1..12: note = Synthetic sequence
GSAGSAAGSGEF

SEQ ID NO: 32 - protein, 143 aa, Homo sapiens
LDSPDRPWNPPTFSPALLVVTEGDNATFTCSFSNTSESFVLNWYRMSPSNQTDKLAAFPEDRSQPGQDCRFRVTQLPNGRDFHMSVVRARRNDSGTYLCGAISLAPKAQIKESLRAELRVTERRAEVPTAHPSPSPRPAGQFQ

SEQ ID NO: 33 - protein, 343 aa, Homo sapiens
EEELQVIQPDKSVLVAAGETATLRCTATSLIPVGPIQWFRGAGPGRELIYNQKEGHFPRVTTVSDLTKRNNMDFSIRIGNITPADAGTYYCVKFRKGSPDDVEFKSGAGTELSVRAKPSAPVVSGPAARATPQHTVSFTCESHGFSPRDITLKWFKNGNELSDFQTNVDPVGESVSYSIHSTAKVVLTREDVHSQVICEVAHVTLQGDPLRGTANLSETIRVPPTLEVTQQPVRAENQVNVTCQVRKFYPQRLQLTWLENGNVSRTETASTVTENKDGTYNWMSWLLVNVSAHRDDVKLTCQVEHDGQPAVSKSHDLKVSAHPKEQGSNTAAENTGSNERNIY

SEQ ID NO: 34 - protein, 127 aa, Homo sapiens
KESCDVQLYIKRQSEHSILAGDPFELECPVKYCANRPHVTWCKLNGTTCVKLEDRQTSWKEEKNISFFILHFEPVLPNDNGSYRCSANFQSNLIESHSTTLYVTDVKSASERPSKDEMASRPWLLYR

SEQ ID NO: 35 - protein, 120 aa, Homo sapiens
MMTGTIETTGNISAEKGGSIILQCHLSSTTAQVTQVNWEQQDQLLAICNADLGWHISPSFKDRVAPGPGLGLTLQSLTVNDTGEYFCIYHTYPDGTYTGRIFLEVLESSVAEHGARFQIP

SEQ ID NO: 36 - protein, 181 aa, Homo sapiens
SEVEYRAEVGQNAYLPCFYTPAAPGNLVPVCWGKGACPVFECGNVVLRTDERDVNYWTSRYWLNGDFRKGDVSLTIENVTLADSGIYCCRIQIPGIMNDEKFNLKLVIKPAKVTPAPTRQRDFTAAFPRMLTTRGHGPAETQTLGSLPDINLTQISTLANELRDSRLANDLRDSGATIRIG

SEQ ID NO: 37 - protein, 202 aa, Homo sapiens
QVQVVTQDEREQLYTPASLKCSLQNAQEALIVTWQKKKAVSPENMVTFSENHGVVIQPAYKDKINITQLGLQNSTITFWNITLEDEGCYMCLFNTFGFGKISGTACLTVYVQPIVSLHYKFSEDHLNITCSATARPAPMVFWKVPRSGIENSTVTLSHPNGTTSVTSILHIKDPKNQVGKEVICQVLHLGTVTDFKQTVNKG

SEQ ID NO: 38 - protein, 128 aa, Homo sapiens
LSVQQGPNLLQVRQGSQATLVCQVDQATAWERLRVKWTKDGAILCQPYITNGSLSLGVCGPQGRLSWQAPSHLTLQLDPVSLNHSGAYVCWAAVEIPELEEAEGNITRLFVDPDDPTQNRNRIASFPG

SEQ ID NO: 39 - protein, 162 aa, Homo sapiens
FKVATPYSLYVCPEGQNVTLTCRLLGPVDKGHDVTFYKTWYRSSRGEVQTCSERRPIRNLTFQDLHLHHGGHQAANTSHDLAQRHGLESASDHHGNFSITMRNLTLLDSGLYCCLVVEIRHHHSEHRVHGAMELQVQTGKDAPSNCVVYPSSSQDSENITAA

SEQ ID NO: 40 - protein, 242 aa, Homo sapiens
VRINGDGQEVLYLAEGDNVRLGCPYVLDPEDYGPNGLDIEWMQVNSDPAHHRENVFLSYQDKRINHGSLPHLQQRVRFAASDPSQYDASINLMNLQVSDTATYECRVKKTTMATRKVIVTVQARPAVPMCWTEGHMTYGNDVVLKCYASGGSQPLSYKWAKISGHHYPYRAGSYTSQHSYHSELSYQESFHSSINQGLNNGDLVLKDISRADDGLYQCTVANNVGYSVCVVEVKVSDSRRIG

SEQ ID NO: 41 - protein, 427 aa, Homo sapiens
EDFRVIGPAHPILAGVGEDALLTCQLLPKRTTMHVEVRWYRSEPSTPVFVHRDGVEVTEMQMEEYRGWVEWIENGIAKGNVALKIHNIQPSDNGQYWCHFQDGNYCGETSLLLKVAGLGSAPSIHMEGPGESGVQLVCTARGWFPEPQVYWEDIRGEKLLAVSEHRIQDKDGLFYAEATLVVRNASAESVSCLVHNPVLTEEKGSVISLPEKLQTELASLKVNGPSQPILVRVGEDIQLTCYLSPKANAQSMEVRWDRSHRYPAVHVYMDGDHVAGEQMAEYRGRTVLVSDAIDEGRLTLQILSARPSDDGQYRCLFEKDDVYQEASLDLKVVSLGSSPLITVEGQEDGEMQPMCSSDGWFPQPHVPWRDMEGKTIPSSSQALTQGSHGLFHVQTLLRVTNISAVDVTCSISIPFLGEEKIATFSLS

SEQ ID NO: 42 - protein, 235 aa, Homo sapiens
LPAQVAFTPYAPEPGSTCRLREYYDQTAQMCCSKCSPGQHAKVFCTKTSDTVCDSCEDSTYTQLWNWVPECLSCGSRCSSDQVETQACTREQNRICTCRPGWYCALSKQEGCRLCAPLRKCRPGFGVARPGTETSDVVCKPCAPGTFSNTTSSTDICRPHQICNVVAIPGNASMDAVCTSTSPTRSMAPGAVHLPQPVSTRSQHTQPTPEPSTAPSTSFLLPMGPSPPAEGSTGD

SEQ ID NO: 43 - protein, 438 aa, Homo sapiens
LEVQVPEDPVVALVGTDATLCCSFSPEPGFSLAQLNLIWQLTDTKQLVHSFAEGQDQGSAYANRTALFPDLLAQGNASLRLQRVRVADEGSFTCFVSIRDFGSAAVSLQVAAPYSKPSMTLEPNKDLRPGDTVTITCSSYQGYPEAEVFWQDGQGVPLTGNVTTSQMANEQGLFDVHSILRVVLGANGTYSCLVRNPVLQQDAHSSVTITPQRSPTGAVEVQVPEDPVVALVGTDATLRCSFSPEPGFSLAQLNLIWQLTDTKQLVHSFTEGRDQGSAYANRTALFPDLLAQGNASLRLQRVRVADEGSFTCFVSIRDFGSAAVSLQVAAPYSKPSMTLEPNKDLRPGDTVTITCSSYRGYPEAEVFWQDGQGVPLTGNVTTSQMANEQGLFDVHSVLRVVLGANGTYSCLVRNPVLQQDAHGSVTITGQPMTFPPEA

SEQ ID NO: 44 - protein, 208 aa, Homo sapiens
CQGSADHVVSISGVPLQLQPNSIQTKVDSIAWKKLLPSQNGFHHILKWENGSLPSNTSNDRFSFIVKNLSLLIKAAQQQDSGLYCLEVTSISGKVQTATFQVFVFESLLPDKVEKPRLQGQGKILDRGRCQVALSCLVSRDGNVSYAWYRGSKLIQTAGNLTYLDEEVDINGTHTYTCNVSNPVSWESHTLNLTQDCQNAHQEFRFWP

SEQ ID NO: 45 - protein, 422 aa, Homo sapiens
VPVVWAQEGAPAQLPCSPTIPLQDLSLLRRAGVTWQHQPDSGPPAAAPGHPLAPGPHPAAPSSWGPRPRRYTVLSVGPGGLRSGRLPLQPRVQLDERGRQRGDFSLWLRPARRADAGEYRAAVHLRDRALSCRLRLRLGQASMTASPPGSLRASDWVILNCSFSRPDRPASVHWFRNRGQGRVPVRESPHHHLAESFLFLPQVSPMDSGPWGCILTYRDGFNVSIMYNLTVLGLEPPTPLTVYAGAGSRVGLPCRLPAGVGTRSFLTAKWTPPGGGPDLLVTGDNGDFTLRLEDVSQAQAGTYTCHIHLQEQQLNATVTLAIITVTPKSFGSPGSLGKLLCEVTPVSGQERFVWSSLDTPSQRSFSGPWLEAQEAQLLSQPWQCQLYQGERLLGAAVYFTELSSPGAQRSGRAPGALPAGHL

SEQ ID NO: 46 - protein, 498 aa, Homo sapiens
IPVIEPSVPELVVKPGATVTLRCVGNGSVEWDGPPSPHWTLYSDGSSSILSTNNATFQNTGTYRCTEPGDPLGGSAAIHLYVKDPARPWNVLAQEVVVFEDQDALLPCLLTDPVLEAGVSLVRVRGRPLMRHTNYSFSPWHGFTIHRAKFIQSQDYQCSALMGGRKVMSISIRLKVQKVIPGPPALTLVPAELVRIRGEAAQIVCSASSVDVNFDVFLQHNNTKLAIPQQSDFHNNRYQKVLTLNLDQVDFQHAGNYSCVASNVQGKHSTSMFFRVVESAYLNLSSEQNLIQEVTVGEGLNLKVMVEAYPGLQGFNWTYLGPFSDHQPEPKLANATTKDTYRHTFTLSLPRLKPSEAGRYSFLARNPGGWRALTFELTLRYPPEVSVIWTFINGSGTLLCAASGYPQPNVTWLQCSGHTDRCDEAQVLQVWDDPYPEVLSQEPFHKVTVQSLLTVETLEHNQTYECRAHNSVGSGSWAFIPISAGAHTHPPDEFLFTP

SEQ ID NO: 47 - protein, 93 aa, Homo sapiens
LQCFCHLCTKDNFTCVTDGLCFVSVTETTDKVIHNSMCIAEIDLIPRDRPFVCAPSSKTGSVTTTYCCNQDHCNKIELPTTVKSSPGLGPVEL

SEQ ID NO: 48 - protein, 214 aa, Homo sapiens
HGTELPSPPSVWFEAEFFHHILHWTPIPNQSESTCYEVALLRYGIESWNSISNCSQTLSYDLTAVTLDLYHSNGYRARVRAVDGSRHSNWTVTNTRFSVDEVTLTVGSVNLEIHNGFILGKIQLPRPKMAPANDTYESIFSHFREYEIAIRKVPGNFTFTHKKVKHENFSLLTSGEVGEFCVQVKPSVASRSNKGMWSKEECISLTRQYFTVTN

SEQ ID NO: 49 - protein, 173 aa, Homo sapiens
EPPTACREKQYLINSQCCSLCQPGQKLVSDCTEFTETECLPCGESEFLDTWNRETHCHQHKYCDPNLGLRVQQKGTSETDTICTCEEGWHCTSEACESCVLHRSCSPGFGVKQIATGVSDTICEPCPVGFFSNVSSAFEKCHPWTSCETKDLVVQQAGTNKTDVVCGPQDRLR

SEQ ID NO: 50 - protein, 186 aa, Homo sapiens [sequence omitted]

SEQ ID NO: 51 - protein, 163 aa, Homo sapiens
LQDPCSNCPAGTFCDNNRNQICSPCPPNSFSSAGGQRTCDICRQCKGVFRTRKECSSTSNAECDCTPGFHCLGAGCSMCEQDCKQGQELTKKGCKDCCFGTFNDQKRGICRPWTNCSLDGKSVLVNGTKERDVVCGPSPADLSPGASSVTPPAPAREPGHSPQ

SEQ ID NO: 52 - protein, 126 aa, Homo sapiens [sequence omitted]

SEQ ID NO: 53 - protein, 220 aa, Homo sapiens
FTVTVPKDLYVVEYGSNMTIECKFPVEKQLDLAALIVYWEMEDKNIIQFVHGEEDLKVQHSSYRQRARLLKDQLSLGNAALQITDVKLQDAGVYRCMISYGGADYKRITVKVNAPYNKINQRILVVDPVTSEHELTCQAEGYPKAEVIWTSSDHQVLSGKTTTTNSKREEKLFNVTSTLRINTTTNEIFYCTFRRLDPEENHTAELVIPELPLAHPPNER

SEQ ID NO: 54 - protein, 201 aa, Homo sapiens
LFTVTVPKELYIIEHGSNVTLECNFDTGSHVNLGAITASLQKVENDTSPHRERATLLEEQLPLGKASFHIPQVQVRDEGQYQCIIIYGVAWDYKYLTLKVKASYRKINTHILKVPETDEVELTCQATGYPLAEVSWPNVSVPANTSHSRTPEGLYQVTSVLRLKPPPGRNFSCVFWNTHVRELTLASIDLQSQMEPRTHPT

SEQ ID NO: 55 - protein, 235 aa, Homo sapiens
LIIGFGISGRHSITVTTVASAGNIGEDGILSCTFEPDIKLSDIVIQWLKEGVLGLVHEFKEGKDELSEQDEMFRGRTAVFADQVIVGNASLRLKNVQLTDAGTYKCYIITSKGKGNANLEYKTGAFSMPEVNVDYNASSETLRCEAPRWFPQPTVVWASQVDQGANFSEVSNTSFELNSENVTMKVVSVLYNVTINNTYSCMIENDIAKATGDIKVTESEIKRRSHLQLLNSKAS

SEQ ID NO: 56 - protein, 133 aa, Homo sapiens
QVSHRYPRIQSIKVQFTEYKKEKGFILTSQKEDEIMKVQNNSVIINCDGFYLISLKGYFSQEVNISLHYQKDEEPLFQLKKVRSVNSLMVASLTYKDKVYLNVTTDNTSLDDFHVNGGELILIHQNPGEFCVL

SEQ ID NO: 57 - protein, 132 aa, Homo sapiens
TSLKPTAIESCMVKFELSSSKWHMTSPKPHCVNTTSDGKLKILQSGTYLIYGQVIPVDKKYIKDNAPFVVQIYKKNDVLQTLMNDFQILPIGGVYELHAGDNIYLKFNSKDHIQKTNTYWGIILMPDLPFIS

SEQ ID NO: 58 - protein, 205 aa, Homo sapiens
ACPWAVSGARASPGSAASPRLREGPELSPDDPAGLLDLRQGMFAQLVAQNVLLIDGPLSWYSDPGLAGVSLTGGLSYKEDTKELVVAKAGVYYVFFQLELRRVVAGEGSGSVSLALHLQPLRSAAGAAALALTVDLPPASSEARNSAFGFQGRLLHLSAGQRLGVHLHTEARARHAWQLTQGATVLGLFRVTPEIPAGLPSPRSE

SEQ ID NO: 59 - protein, 195 aa, Homo sapiens
SQLRAQGEACVQFQALKGQEFAPSHQQVYAPLRADGDKPRAHLTVVRQTPTQHFKNQFPALHWEHELGLAFTKNRMNYTNKFLLIPESGDYFIYSQVTFRGMTSECSEIRQAGRPNKPDSITVVITKVTDSYPEPTQLLMGTKSVCEVGSNWFQPIYLGAMFSLQEGDKLMVNVSDISLVDYTKEDKTFFGAFLL

SEQ ID NO: 60 - protein, 215 aa, Homo sapiens
HRRLDKIEDERNLHEDFVFMKTIQRCNTGERSLSLLNCEEIKSQFEGFVKDIMLNKEETKKENSFEMQKGDQNPQIAAHVISEASSKTTSVLQWAEKGYYTMSNNLVTLENGKQLTVKRQGLYYIYAQVTFCSNREASSQAPFIASLCLKSPGRFERILLRAANTHSSAKPCGQQSIHLGGVFELQPGASVFVNVTDPSQVSHGTGFTSFGLLKL

SEQ ID NO: 61 - protein, 172 aa, Homo sapiens
QRTDSIPNSPDNVPLKGGNCSEDLLCILKRAPFKKSWAYLQVAKHLNKTKLSWNKDGILHGVRYQDGNLVIQFPGLYFIICQLQFLVQCPNNSVDLKLELLINKHIKKQALVTVCESGMQTKHVYQNLSQFLLDYLQVNTTISVNVDTFQYIDTSTFPLENVLSIFLYSNSD

SEQ ID NO: 62 - protein, 243 aa, Homo sapiens
TNELKQMQDKYSKSGIACFLKEDDSYWDPNDEESMNSPCWQVKWQLRQLVRKMILRTSEETISTVQEKQQNISPLVRERGPQRVAAHITGTRGRSNTLSSPNSKNEKALGRKINSWESSRSGHSFLSNLHLRNGELVIHEKGFYYIYSQTYFRFQEEIKENTKNDKQMVQYIYKYTSYPDPILLMKSARNSCWSKDAEYGLYSIYQGGIFELKENDRIFVSVTNEHLIDMDHEASFFGAFLVG

SEQ ID NO: 63 - protein, 155 aa, Homo sapiens
QRFAQAQQQLPLESLGWDVAELQLNHTGPQQDPRLYWQGGPALGRSFLHGPELDKGQLRIHRDGIYMVHIQVTLAICSSTTASRHHPTTLAVGICSPASRSISLLRLSFHQGCTIASQRLTPLARGDTLCTNLTGTLLPSRNTDETFFGVQWVRP

SEQ ID NO: 64-69 - skipped (6 entries)

SEQ ID NO: 70 - protein, 217 aa, synthetic construct
  REGION 1..217: note = Synthetic sequence
APEFLGGPSVFLFPPKPKDTLMISRTPEVTCVVVDVSQEDPEVQFNWYVDGVEVHNAKTKPREEQFNSTYRVVSVLTVLHQDWLSGKEYKCKVSSKGLPSSIEKTISNATGQPREPQVYTLPPSQEEMTKNQVSLTCLVKGFYPSDIAVEWESNGQPENNYKTTPPVLDSDGSFFLYSRLTVDKSSWQEGNVFSCSVMHEALHNHYTQKSLSLSLGK

SEQ ID NO: 71 - protein, 217 aa, synthetic construct; identical to SEQ ID NO: 70
  REGION 1..217: note = Synthetic sequence

SEQ ID NO: 72 - protein, 217 aa, synthetic construct
  REGION 1..217: note = Synthetic sequence
APEFLGGPSVFLFPPKPKDQLMISRTPEVTCVVVDVSQEDPEVQFNWYVDGVEVHNAKTKPREEQFNSTYRVVSVLTTPHSDWLSGKEYKCKVSSKGLPSSIEKTISNATGQPREPQVYTLPPSQEEMTKNQVSLTCLVKGFYPSDIAVEWESNGQPENNYKTTPPVLDSDGSFFLYSRLTVDKSSWQEGNVFSCSVLHEALHNHYTQKSLSLSLGK

SEQ ID NO: 73 - protein, 11 aa, synthetic construct
  REGION 1..11: note = Synthetic sequence
SKYGPPCPSCP

SEQ ID NO: 74 - protein, 11 aa, synthetic construct
  REGION 1..11: note = Synthetic sequence
SKYGPPCPPCP

SEQ ID NO: 75 - protein, 6 aa, synthetic construct
  REGION 1..6: note = Synthetic sequence
SKYGPP

SEQ ID NO: 76 - protein, 6 aa, synthetic construct
  REGION 1..6: note = Synthetic sequence
IEGRMD

SEQ ID NO: 77 - protein, 9 aa, synthetic construct
  REGION 1..9: note = Synthetic sequence
GGGVPRDCG

SEQ ID NO: 78 - protein, 15 aa, synthetic construct
  REGION 1..15: note = Synthetic sequence
IEGRMDGGGGAGGGG